European Patent Specification EP 3 800 193 B1, published January 11, 2023. Title: PEPTIDE HAVING SKIN-WHITENING ACTIVITY AND USE THEREOF. Applicant: CAREGEN CO., LTD. The sequence listing filed with the application follows.

SEQUENCE LISTING (17 sequences)

SEQ ID NO: 1 - protein, 11 aa, Artificial Sequence
  Peptide 1
LRKRKRRFWVL

SEQ ID NO: 2 - protein, 7 aa, Artificial Sequence
  Peptide 2
FHFIPNW

SEQ ID NO: 3 - protein, 6 aa, Artificial Sequence
  Peptide 3
WPFLRP

SEQ ID NO: 4 - DNA, 20 bp, Artificial Sequence
  Rab27a_F
gaaaatagcgccaagcaccc

SEQ ID NO: 5 - DNA, 20 bp, Artificial Sequence
  Rab27a_R
cctctttcactgccctctgg

SEQ ID NO: 6 - DNA, 20 bp, Artificial Sequence
  Mlph_F
acgatgtcaggggcaaacat

SEQ ID NO: 7 - DNA, 20 bp, Artificial Sequence
  Mlph_R
ctcctctgtgtcagcactgg

SEQ ID NO: 8 - DNA, 20 bp, Artificial Sequence
  myosin VA_F
ttctacattgtgggcgccat

SEQ ID NO: 9 - DNA, 20 bp, Artificial Sequence
  myosin VA_R
tcctccaggttggtcaatcg

SEQ ID NO: 10 - DNA, 21 bp, Artificial Sequence
  MITF_F
ccagcctggcgatcatgtcat

SEQ ID NO: 11 - DNA, 20 bp, Artificial Sequence
  MITF_R
ggtctggacaggagttgctg

SEQ ID NO: 12 - DNA, 20 bp, Artificial Sequence
  Tyrosinase_F
ggccagctttcaggcagagg

SEQ ID NO: 13 - DNA, 20 bp, Artificial Sequence
  Tyrosinase_R
tggtgcttcatgggcaaaat

SEQ ID NO: 14 - DNA, 20 bp, Artificial Sequence
  TRP1_F
tctgtgaaggtgtgcaggag

SEQ ID NO: 15 - DNA, 20 bp, Artificial Sequence
  TRP1_R
ccgaaacagagtggaaggtt

SEQ ID NO: 16 - DNA, 25 bp, Artificial Sequence
  GAPDH_F
ggtgtgaacggatttggccgtattg

SEQ ID NO: 17 - DNA, 25 bp, Artificial Sequence
  GAPDH_R
ccgttgaatttgccgtgagtggagt